European Patent Application EP 4 410 994 A1, published August 7, 2024. Title: NUCLEIC ACID AMPLIFICATION-PROMOTING AGENT AND TEST METHOD USING SAME. Applicant: NOF CORPORATION. Application EP 22 876 206.8, filed September 27, 2022. The sequence listing filed with the application follows.

SEQUENCE LISTING (2 sequences)

SEQ ID NO: 1 - DNA, 25 bp, synthetic construct
  source 1..25: PCR_primers = fwd_seq: cagccgcgctggatgaactgatacc, rev_seq: agcggagacgggcaatcagttcatc; mol_type = other DNA
cagccgcgctggatgaactgatacc

SEQ ID NO: 2 - DNA, 25 bp, synthetic construct
  misc_feature 1..25: note = Reverse Primer
  source 1..25: mol_type = other DNA
agcggagacgggcaatcagttcatc